European Patent Application EP 4 606 385 A1, published August 27, 2025. Title: An agent for treating T-cell tumor. Applicant: Meiji Seika Pharma Co., Ltd. Application WO. The sequence listing filed with the application follows.

SEQUENCE LISTING (143 sequences)

SEQ ID NO: 1 - protein, 485 aa, synthetic construct
  source 1..485: note = CCR0001 VH
EVQLVESGGDLVQPGRSLRLSCAASGFIFSNYGMSWVRQAPGKGLEWVATISSASTYSYYPDSVKGRFTISRDNAKNSLYLQMNSLRVEDTALYYCGRHSDGNFAFGYWGQGTLVTVSSASTKGPSVFPLAPSSKSTSGGTAALGCLVKDYFPEPVTVSWNSGALTSGVHTFPAVLQSSGLYSLSSVVTVPSSSLGTQTYICNVNHKPSNTKVDKRVEPKSCGGGGSEVRLQQSGPDLIKPGASVKMSCKASGYTFTGYVMHWVKQRPGQGLEWIGFINPYNDDIQSNERFRGKATLTSDKSSTTAYMELSSLTSEDSAVYYCARGAGYNFDGAYRFFDFWGQGTTLTVSSGGGGSGGGGSGGGGSDVVMTQSPLSLPVSLGDQASISCRSSQRLVHSNGNTYLHWYLQKPGQSPKLLIYRVSNRFPGVPDRFSGSGSGTDFTLKISRVEAEDLGIYFCSQSTHVPYTFGGGTKLEIKRHHHHHH

SEQ ID NO: 2 - protein, 219 aa, synthetic construct
  source 1..219: note = CCR0001 VL
DVLMTQSPLSLPVTPGEPASISCRSSRNIVHINGDTYLEWYLQKPGQSPQLLIYKVSNRFSGVPDRFSGSGSGTDFTLKISRVEAEDVGVYYCFQGSLLPWTFGQGTKVEIKRTVAAPSVFIFPPSDEQLKSGTASVVCLLNNFYPREAKVQWKVDNALQSGNSQESVTEQDSKDSTYSLSSTLTLSKADYEKHKVYACEVTHQGLSSPVTKSFNRGEC

SEQ ID NO: 3 - protein, 706 aa, synthetic construct
  source 1..706: note = CCR0004 VH
EVQLVESGGDLVQPGRSLRLSCAASGFIFSNYGMSWVRQAPGKGLEWVATISSASTYSYYPDSVKGRFTISRDNAKNSLYLQMNSLRVEDTALYYCGRHSDGNFAFGYWGQGTLVTVSSASTKGPSVFPLAPSSKSTSGGTAALGCLVKDYFPEPVTVSWNSGALTSGVHTFPAVLQSSGLYSLSSVVTVPSSSLGTQTYICNVNHKPSNTKVDKRVEPKSCGGGGSEVRLQQSGPDLIKPGASVKMSCKASGYTFTGYVMHWVKQRPGQGLEWIGFINPYNDDIQSNERFRGKATLTSDKSSTTAYMELSSLTSEDSAVYYCARGAGYNFDGAYRFFDFWGQGTTLTVSSGGGGSGGGGSGGGGSDVVMTQSPLSLPVSLGDQASISCRSSQRLVHSNGNTYLHWYLQKPGQSPKLLIYRVSNRFPGVPDRFSGSGSGTDFTLKISRVEAEDLGIYFCSQSTHVPYTFGGGTKLEIKRDKTHTCPPCPAPEAAGGPSVFLFPPKPKDTLMISRTPEVTCVVVDVSHEDPEVKFNWYVDGVEVHNAKTKPREEQYNSTYRVVSVLTVLHQDWLNGKEYKCKVSNKALPAPIEKTISKAKGQPREPQVYTLPPSREEMTKNQVSLTCLVKGFYPSDIAVEWESNGQPENNYKTTPPVLDSDGSFFLYSKLTVDKSRWQQGNVFSCSVMHEALHNHYTQKSLSLSPGK

SEQ ID NO: 4 - protein, 124 aa, synthetic construct
  source 1..124: note = anti-TRBC-1 antibody VH
EVRLQQSGPDLIKPGASVKMSCKASGYTFTGYVMHWVKQRPGQGLEWIGFINPYNDDIQSNERFRGKATLTSDKSSTTAYMELSSLTSEDSAVYYCARGAGYNFDGAYRFFDFWGQGTTLTVSS

SEQ ID NO: 5 - protein, 113 aa, synthetic construct
  source 1..113: note = anti-TRBC-1 antibody VL
DVVMTQSPLSLPVSLGDQASISCRSSQRLVHSNGNTYLHWYLQKPGQSPKLLIYRVSNRFPGVPDRFSGSGSGTDFTLKISRVEAEDLGIYFCSQSTHVPYTFGGGTKLEIKR

SEQ ID NO: 6 - protein, 124 aa, synthetic construct
  source 1..124: note = anti-TRBC-2 antibody VH
QVQLVQSGAEVKKPGASVKVSCKASGYKFTGFVMHWVRQAPGQGLEWMGFINPYNDDIQSNERFRGRVTMTRDTSISTAYMELSRLRSDDTAVYYCARGNGYNFDGAYRFFDFWGQGTMVTVSS

SEQ ID NO: 7 - protein, 112 aa, synthetic construct
  source 1..112: note = anti-TRBC-2 antibody VL
DIVMTQSPLSLPVTPGEPASISCRSSQRLVHSNGNTYLHWYLQKPGQSPRLLIYRVSNRFPGVPDRFSGSGSGTDFTLKISRVEAEDVGVYYCSQSTHVPYTFGQGTKLEIK

SEQ ID NO: 8 - protein, 119 aa, synthetic construct
  source 1..119: note = anti-CCR4 antibody VH
EVQLVESGGDLVQPGRSLRLSCAASGFIFSNYGMSWVRQAPGKGLEWVATISSASTYSYYPDSVKGRFTISRDNAKNSLYLQMNSLRVEDTALYYCGRHSDGNFAFGYWGQGTLVTVSS

SEQ ID NO: 9 - protein, 112 aa, synthetic construct
  source 1..112: note = anti-CCR4 antibody VL
DVLMTQSPLSLPVTPGEPASISCRSSRNIVHINGDTYLEWYLQKPGQSPQLLIYKVSNRFSGVPDRFSGSGSGTDFTLKISRVEAEDVGVYYCFQGSLLPWTFGQGTKVEIK

SEQ ID NO: 10 - protein, 5 aa, synthetic construct
  source 1..5: note = anti-TRBC-1 antibody VH CDR1
GYVMH

SEQ ID NO: 11 - protein, 17 aa, synthetic construct
  source 1..17: note = anti-TRBC-1 antibody VH CDR2
FINPYNDDIQSNERFRG

SEQ ID NO: 12 - protein, 15 aa, synthetic construct
  source 1..15: note = anti-TRBC-1 antibody VH CDR3
GAGYNFDGAYRFFDF

SEQ ID NO: 13 - protein, 16 aa, synthetic construct
  source 1..16: note = anti-TRBC-1 antibody VL CDR1
RSSQRLVHSNGNTYLH

SEQ ID NO: 14 - protein, 7 aa, synthetic construct
  source 1..7: note = anti-TRBC-1 antibody VL CDR2
RVSNRFP

SEQ ID NO: 15 - protein, 9 aa, synthetic construct
  source 1..9: note = anti-TRBC-1 antibody VL CDR3
SQSTHVPYT

SEQ ID NO: 16 - protein, 5 aa, synthetic construct
  source 1..5: note = anti-TRBC-2 antibody VH CDR1
GFVMH

SEQ ID NO: 17 - protein, 17 aa, synthetic construct
  source 1..17: note = anti-TRBC-2 antibody VH CDR2
FINPYNDDIQSNERFRG

SEQ ID NO: 18 - protein, 15 aa, synthetic construct
  source 1..15: note = anti-TRBC-2 antibody VH CDR3
GNGYNFDGAYRFFDF

SEQ ID NO: 19 - protein, 16 aa, synthetic construct
  source 1..16: note = anti-TRBC-2 antibody VL CDR1
RSSQRLVHSNGNTYLH

SEQ ID NO: 20 - protein, 7 aa, synthetic construct
  source 1..7: note = anti-TRBC-2 antibody VL CDR2
RVSNRFP

SEQ ID NO: 21 - protein, 9 aa, synthetic construct
  source 1..9: note = anti-TRBC-2 antibody VL CDR3
SQSTHVPYT

SEQ ID NO: 22 - protein, 5 aa, synthetic construct
  source 1..5: note = anti-CCR4 antibody VH CDR1
NYGMS

SEQ ID NO: 23 - protein, 17 aa, synthetic construct
  source 1..17: note = anti-CCR4 antibody VH CDR2
TISSASTYSYYPDSVKG

SEQ ID NO: 24 - protein, 10 aa, synthetic construct
  source 1..10: note = anti-CCR4 antibody VH CDR3
HSDGNFAFGY

SEQ ID NO: 25 - protein, 16 aa, synthetic construct
  source 1..16: note = anti-CCR4 antibody VL CDR1
RSSRNIVHINGDTYLE

SEQ ID NO: 26 - protein, 7 aa, synthetic construct
  source 1..7: note = anti-CCR4 antibody VL CDR2
KVSNRFS

SEQ ID NO: 27 - protein, 9 aa, synthetic construct
  source 1..9: note = anti-CCR4 antibody VL CDR3
FQGSLLPWT

SEQ ID NO: 28 - protein, 484 aa, synthetic construct
  source 1..484: note = CCR0010 VH
EVQLVESGGDLVQPGRSLRLSCAASGFIFSNYGMSWVRQAPGKGLEWVATISSASTYSYYPDSVKGRFTISRDNAKNSLYLQMNSLRVEDTALYYCGRHSDGNFAFGYWGQGTLVTVSSASTKGPSVFPLAPSSKSTSGGTAALGCLVKDYFPEPVTVSWNSGALTSGVHTFPAVLQSSGLYSLSSVVTVPSSSLGTQTYICNVNHKPSNTKVDKRVEPKSCGGGGSQVQLVQSGAEVKKPGASVKVSCKASGYKFTGFVMHWVRQAPGQGLEWMGFINPYNDDIQSNERFRGRVTMTRDTSISTAYMELSRLRSDDTAVYYCARGNGYNFDGAYRFFDFWGQGTMVTVSSGGGGSGGGGSGGGGSDIVMTQSPLSLPVTPGEPASISCRSSQRLVHSNGNTYLHWYLQKPGQSPRLLIYRVSNRFPGVPDRFSGSGSGTDFTLKISRVEAEDVGVYYCSQSTHVPYTFGQGTKLEIKHHHHHH

SEQ ID NO: 29 - protein, 214 aa, synthetic construct
  source 1..214: note = CD1a1001 VL
DIQMTQSPSSLSASVGDRVTITCRASQSISSYLNWYQQKPGKAPKLLIYAASSLQSGVPSRFSGSGSGTDFTLTISSLQPEDFATYYCQQSYSTPPTFGQGTKVEIKRTVAAPSVFIFPPSDEQLKSGTASVVCLLNNFYPREAKVQWKVDNALQSGNSQESVTEQDSKDSTYSLSSTLTLSKADYEKHKVYACEVTHQGLSSPVTKSFNRGEC

SEQ ID NO: 30 - protein, 483 aa, synthetic construct
  source 1..483: note = CD1a1001 VH
QVQLQESGAGLLKPSETLSLTCAVYGGSFSGYYWSWIRQPPGKGLEWIGYIYYSGSTNYNPSLKSRVTISVDTSKNQFSLKLSSVTAADTAVYYCAKAPYMMYFDSWGQGTLVTVSSASTKGPSVFPLAPSSKSTSGGTAALGCLVKDYFPEPVTVSWNSGALTSGVHTFPAVLQSSGLYSLSSVVTVPSSSLGTQTYICNVNHKPSNTKVDKRVEPKSCGGGGSEVRLQQSGPDLIKPGASVKMSCKASGYTFTGYVMHWVKQRPGQGLEWIGFINPYNDDIQSNERFRGKATLTSDKSSTTAYMELSSLTSEDSAVYYCARGAGYNFDGAYRFFDFWGQGTTLTVSSGGGGSGGGGSGGGGSDVVMTQSPLSLPVSLGDQASISCRSSQRLVHSNGNTYLHWYLQKPGQSPKLLIYRVSNRFPGVPDRFSGSGSGTDFTLKISRVEAEDLGIYFCSQSTHVPYTFGGGTKLEIKRHHHHHH

SEQ ID NO: 31 - protein, 482 aa, synthetic construct
  source 1..482: note = CD1a1003 VH
QVQLQESGAGLLKPSETLSLTCAVYGGSFSGYYWSWIRQPPGKGLEWIGYIYYSGSTNYNPSLKSRVTISVDTSKNQFSLKLSSVTAADTAVYYCAKAPYMMYFDSWGQGTLVTVSSASTKGPSVFPLAPSSKSTSGGTAALGCLVKDYFPEPVTVSWNSGALTSGVHTFPAVLQSSGLYSLSSVVTVPSSSLGTQTYICNVNHKPSNTKVDKRVEPKSCGGGGSQVQLVQSGAEVKKPGASVKVSCKASGYKFTGFVMHWVRQAPGQGLEWMGFINPYNDDIQSNERFRGRVTMTRDTSISTAYMELSRLRSDDTAVYYCARGNGYNFDGAYRFFDFWGQGTMVTVSSGGGGSGGGGSGGGGSDIVMTQSPLSLPVTPGEPASISCRSSQRLVHSNGNTYLHWYLQKPGQSPRLLIYRVSNRFPGVPDRFSGSGSGTDFTLKISRVEAEDVGVYYCSQSTHVPYTFGQGTKLEIKHHHHHH

SEQ ID NO: 32 - protein, 704 aa, synthetic construct
  source 1..704: note = CD1a1004 VH
QVQLQESGAGLLKPSETLSLTCAVYGGSFSGYYWSWIRQPPGKGLEWIGYIYYSGSTNYNPSLKSRVTISVDTSKNQFSLKLSSVTAADTAVYYCAKAPYMMYFDSWGQGTLVTVSSASTKGPSVFPLAPSSKSTSGGTAALGCLVKDYFPEPVTVSWNSGALTSGVHTFPAVLQSSGLYSLSSVVTVPSSSLGTQTYICNVNHKPSNTKVDKRVEPKSCGGGGSEVRLQQSGPDLIKPGASVKMSCKASGYTFTGYVMHWVKQRPGQGLEWIGFINPYNDDIQSNERFRGKATLTSDKSSTTAYMELSSLTSEDSAVYYCARGAGYNFDGAYRFFDFWGQGTTLTVSSGGGGSGGGGSGGGGSDVVMTQSPLSLPVSLGDQASISCRSSQRLVHSNGNTYLHWYLQKPGQSPKLLIYRVSNRFPGVPDRFSGSGSGTDFTLKISRVEAEDLGIYFCSQSTHVPYTFGGGTKLEIKRDKTHTCPPCPAPEAAGGPSVFLFPPKPKDTLMISRTPEVTCVVVDVSHEDPEVKFNWYVDGVEVHNAKTKPREEQYNSTYRVVSVLTVLHQDWLNGKEYKCKVSNKALPAPIEKTISKAKGQPREPQVYTLPPSREEMTKNQVSLTCLVKGFYPSDIAVEWESNGQPENNYKTTPPVLDSDGSFFLYSKLTVDKSRWQQGNVFSCSVMHEALHNHYTQKSLSLSPGK

SEQ ID NO: 33 - protein, 703 aa, synthetic construct
  source 1..703: note = CD1a1006 VH
QVQLQESGAGLLKPSETLSLTCAVYGGSFSGYYWSWIRQPPGKGLEWIGYIYYSGSTNYNPSLKSRVTISVDTSKNQFSLKLSSVTAADTAVYYCAKAPYMMYFDSWGQGTLVTVSSASTKGPSVFPLAPSSKSTSGGTAALGCLVKDYFPEPVTVSWNSGALTSGVHTFPAVLQSSGLYSLSSVVTVPSSSLGTQTYICNVNHKPSNTKVDKRVEPKSCGGGGSQVQLVQSGAEVKKPGASVKVSCKASGYKFTGFVMHWVRQAPGQGLEWMGFINPYNDDIQSNERFRGRVTMTRDTSISTAYMELSRLRSDDTAVYYCARGNGYNFDGAYRFFDFWGQGTMVTVSSGGGGSGGGGSGGGGSDIVMTQSPLSLPVTPGEPASISCRSSQRLVHSNGNTYLHWYLQKPGQSPRLLIYRVSNRFPGVPDRFSGSGSGTDFTLKISRVEAEDVGVYYCSQSTHVPYTFGQGTKLEIKDKTHTCPPCPAPEAAGGPSVFLFPPKPKDTLMISRTPEVTCVVVDVSHEDPEVKFNWYVDGVEVHNAKTKPREEQYNSTYRVVSVLTVLHQDWLNGKEYKCKVSNKALPAPIEKTISKAKGQPREPQVYTLPPSREEMTKNQVSLTCLVKGFYPSDIAVEWESNGQPENNYKTTPPVLDSDGSFFLYSKLTVDKSRWQQGNVFSCSVMHEALHNHYTQKSLSLSPGK

SEQ ID NO: 34 - protein, 4 aa, synthetic construct
  source 1..4: note = anti-CD1a antibody VH CDR1
GYYW

SEQ ID NO: 35 - protein, 16 aa, synthetic construct
  source 1..16: note = anti-CD1a antibody VH CDR2
YIYYSGSTNYNPSLKS

SEQ ID NO: 36 - protein, 9 aa, synthetic construct
  source 1..9: note = anti-CD1a antibody VH CDR3
APYMMYFDS

SEQ ID NO: 37 - protein, 11 aa, synthetic construct
  source 1..11: note = anti-CD1a antibody VL CDR1
RASQSISSYLN

SEQ ID NO: 38 - protein, 7 aa, synthetic construct
  source 1..7: note = anti-CD1a antibody VL CDR2
AASSLQS

SEQ ID NO: 39 - protein, 9 aa, synthetic construct
  source 1..9: note = anti-CD1a antibody VL CDR3
QQSYSTPPT

SEQ ID NO: 40 - protein, 117 aa, synthetic construct
  source 1..117: note = anti-CD1a antibody VH
QVQLQESGAGLLKPSETLSLTCAVYGGSFSGYYWSWIRQPPGKGLEWIGYIYYSGSTNYNPSLKSRVTISVDTSKNQFSLKLSSVTAADTAVYYCAKAPYMMYFDSWGQGTLVTVSS

SEQ ID NO: 41 - protein, 107 aa, synthetic construct
  source 1..107: note = anti-CD1a antibody VL
DIQMTQSPSSLSASVGDRVTITCRASQSISSYLNWYQQKPGKAPKLLIYAASSLQSGVPSRFSGSGSGTDFTLTISSLQPEDFATYYCQQSYSTPPTFGQGTKVEIK

SEQ ID NO: 42 - DNA, 1455 bp, synthetic construct
  source 1..1455: mol_type = other DNA; note = Nucleotide sequence encoding CCR0001 VH (SEQ ID NO:1)
gaagtgcagctggtcgagtctggaggagatctggtgcaacctggccgttcccttcgattgtcatgtgcagcatccgggttcatcttctccaactacggtatgagctgggtcagacaagcacccggaaaaggccttgaatgggttgccacaatctcctctgccagtacctactcttattaccccgacagcgtaaagggtcgattcaccattagccgggacaatgctaagaactcactctacctccagatgaacagcctgagggtggaggacaccgctctgtactattgcggcagacacagtgacggtaatttcgcctttgggtattggggtcaaggaaccctggttactgtctcctctgcatctaccaagggtcccagcgtgtttcccctggctccatcctccaaaagcacgagcggcggaacagcagccttaggttgcctcgtaaaagactactttcccgagccggtgacagtctcctggaactcgggagctctgacatccggagtgcataccttccctgctgtcctgcagagttctggcctctacagcctctcctctgtcgtcacagttccttcatccagcttggggacccagacatacatctgcaacgtcaatcacaaacccagcaatacaaaggtagacaaacgggtggagccgaaatcctgtgggggcgggggatccgaggtgaggttacagcaaagtggcccagacctgattaagcccggtgccagcgttaagatgtcatgcaaggcgtctgggtatacctttaccggttacgtcatgcattgggtcaagcaaagacccggccagggtttggagtggataggcttcatcaacccttataacgatgacattcagtctaatgagcgcttccgagggaaagccacacttaccagcgataagtcaagcactactgcctacatggagctgagctctctgactagtgaagactctgccgtgtattactgtgccagaggagccgggtataatttcgacggagcataccggtttttcgatttctggggtcagggcacaaccctgacggtgagttctgggggagggggctcaggtggaggaggctctgggggcggaggcagtgatgtggtgatgacccaatcccctcttagtctgcctgtgagcttaggcgatcaagcctccatctcttgtcgcagttcccagcgactggttcacagtaacggcaatacctacttgcactggtaccttcagaaaccagggcaaagtcccaagctattgatttaccgtgtctcgaatcggtttccaggcgttcctgaccgttttagcggaagcggttctggaactgactttacactcaagatctcccgagtggaggcggaagacttgggcatctatttctgctcacagagtacacatgtcccctataccttcggtggggggactaagctcgaaatcaagcggcatcaccaccatcaccat

SEQ ID NO: 43 - DNA, 657 bp, synthetic construct
  source 1..657: mol_type = other DNA; note = Nucleotide sequence encoding CCR0001 VL [SEQ ID NO:2]
gatgtgctgatgacgcagagtccccttagcctgcctgtgactcctggggaacccgcttccatttcctgtcggagctcaaggaacatagtccacatcaatggcgatacctatctggagtggtatctgcagaaaccaggccagtctccacagttgctgatctacaaagtgagcaatcggtttagcggcgtgcctgatcgcttttctgggtctgggagtgggacagacttcaccctgaagatctcaagggttgaagccgaggatgtaggggtgtattactgcttccagggctcattgctcccatggacatttggacagggcactaaggtggagattaagcgaacagtggctgctccttctgtgttcatctttccacccagcgacgaacagctgaagtctggaactgcctctgttgtgtgtctcctgaacaacttctatcccagagaagccaaggtacagtggaaagtggacaatgcgttgcagagtggcaactcccaggagagcgttactgagcaggatagcaaggacagtacctactccttgagctccacgctgacccttagcaaagccgattacgagaagcacaaggtctatgcgtgcgaagtcactcaccaaggcctgtcaagtccagtgaccaagtctttcaatcgtggggaatgc

SEQ ID NO: 44 - DNA, 2118 bp, synthetic construct
  source 1..2118: mol_type = other DNA; note = Nucleotide sequence encoding CCR0004 VH (SEQ ID NO:3)
gaagtgcagctggtcgagtctggaggagatctggtgcaacctggccgttcccttcgattgtcatgtgcagcatccgggttcatcttctccaactacggtatgagctgggtcagacaagcacccggaaaaggccttgaatgggttgccacaatctcctctgccagtacctactcttattaccccgacagcgtaaagggtcgattcaccattagccgggacaatgctaagaactcactctacctccagatgaacagcctgagggtggaggacaccgctctgtactattgcggcagacacagtgacggtaatttcgcctttgggtattggggtcaaggaaccctggttactgtctcctctgcatctaccaagggtcccagcgtgtttcccctggctccatcctccaaaagcacgagcggcggaacagcagccttaggttgcctcgtaaaagactactttcccgagccggtgacagtctcctggaactcgggagctctgacatccggagtgcataccttccctgctgtcctgcagagttctggcctctacagcctctcctctgtcgtcacagttccttcatccagcttggggacccagacatacatctgcaacgtcaatcacaaacccagcaatacaaaggtagacaaacgggtggagccgaaatcctgtgggggcgggggatccgaggtgaggttacagcaaagtggcccagacctgattaagcccggtgccagcgttaagatgtcatgcaaggcgtctgggtatacctttaccggttacgtcatgcattgggtcaagcaaagacccggccagggtttggagtggataggcttcatcaacccttataacgatgacattcagtctaatgagcgcttccgagggaaagccacacttaccagcgataagtcaagcactactgcctacatggagctgagctctctgactagtgaagactctgccgtgtattactgtgccagaggagccgggtataatttcgacggagcataccggtttttcgatttctggggtcagggcacaaccctgacggtgagttctgggggagggggctcaggtggaggaggctctgggggcggaggcagtgatgtggtgatgacccaatcccctcttagtctgcctgtgagcttaggcgatcaagcctccatctcttgtcgcagttcccagcgactggttcacagtaacggcaatacctacttgcactggtaccttcagaaaccagggcaaagtcccaagctattgatttaccgtgtctcgaatcggtttccaggcgttcctgaccgttttagcggaagcggttctggaactgactttacactcaagatctcccgagtggaggcggaagacttgggcatctatttctgctcacagagtacacatgtcccctataccttcggtggggggactaagctcgaaatcaagcgggataagactcacacgtgtcccccatgtccagcccctgaagccgcaggcggtccatcagttttcctgtttccccctaagcccaaagacaccctcatgatctcgaggactcctgaggtgacttgcgtagtggtagacgtgagtcatgaagatcccgaagtgaagttcaactggtatgtcgacggcgtagaagtgcacaatgccaagacaaagcccagggaagaacagtacaactccacctatagagttgtttccgtattgactgtgctgcatcaggactggctaaatgggaaggaatacaaatgcaaagtctccaacaaagctcttcctgcccccattgagaagaccatctcgaaagctaaaggccaacctagggaaccacaggtttatacgttaccgcctagcagggaggagatgactaaaaatcaggtgtctctgacatgtctcgtgaaaggcttttacccatcagacattgcggttgagtgggagtctaatggacagccggagaataactacaagacaactcctcccgtgctggattccgatggctcattctttctgtactcaaaactcactgtggacaagtcacgctggcagcaggggaacgttttctcctgcagtgtgatgcacgaggctcttcacaaccactatacacagaagtcactgtctctgagcccaggtaaa

SEQ ID NO: 45 - DNA, 1452 bp, synthetic construct
  source 1..1452: mol_type = other DNA; note = Nucleotide sequence encoding CCR0010 VH (SEQ ID NO:28)
gaagtgcagctggtcgagtctggaggagatctggtgcaacctggccgttcccttcgattgtcatgtgcagcatccgggttcatcttctccaactacggtatgagctgggtcagacaagcacccggaaaaggccttgaatgggttgccacaatctcctctgccagtacctactcttattaccccgacagcgtaaagggtcgattcaccattagccgggacaatgctaagaactcactctacctccagatgaacagcctgagggtggaggacaccgctctgtactattgcggcagacacagtgacggtaatttcgcctttgggtattggggtcaaggaaccctggttactgtctcctctgccagcacaaagggccccagcgtctttccgttagctcccagttcaaagtctactagtggtggtaccgcagctctgggctgtctggtcaaggactacttcccagaaccggtgactgtatcttggaatagcggggctcttactagcggagtgcacacttttcccgcagtccttcagtcctcaggattatacagtctcagcagtgttgttaccgtgcctagctccagtttgggcacgcaaacgtatatctgcaatgtcaaccataaaccttccaatacgaaagtggacaaacgagtggaaccaaagtcctgtgggggcgggggatcccaggttcagctcgtacagagtggagctgaagtcaagaaaccaggtgcatcagtcaaggtgtcctgcaaagcttcagggtataagtttacagggttcgtgatgcactgggtgagacaggctcctggacaaggcctggaatggatgggcttcatcaacccctacaatgacgacatccagtccaatgagcgatttcgtggtagggtgacgatgacacgggatacctccattagcactgcctatatggagctgtctcgcttgaggagtgacgatactgccgtttactactgtgccagaggtaacggctacaacttcgatggggcctatcggttcttcgacttttggggacaaggcaccatggtcacagtgtctagcggaggaggcgggtcaggaggaggagggtctggcggcggtggctctgacattgtgatgactcagtcacccctttctctgcccgttactcctggagaaccagccagcatatcctgccgttctagccagaggttggtgcactccaatgggaacacctatctgcactggtatctccagaaaccaggacagagtcctagactgctgatctaccgagtcagcaaccgctttccaggtgttcctgatcggttctcaggttctgggagtggcacagacttcacgctcaagatctccagggtcgaagctgaggatgtaggcgtgtactactgtagccagtccacacatgtgccctatacctttggacaaggcaccaaactggagattaagcatcaccaccatcaccat

SEQ ID NO: 46 - DNA, 1449 bp, synthetic construct
  source 1..1449: mol_type = other DNA; note = Nucleotide sequence encoding CD1a1001 VH
caggtacagttgcaggaatctggcgctggattgctgaagccatccgagactctgagcctgacatgtgccgtctatggtggctccttttccgggtattactggagctggattcggcaacctcctggcaaagggcttgagtggataggctacatctactattccggaagcaccaactacaatccctcactcaagagtagggtcaccatcagtgtggacacgtctaagaaccagttctccctgaagctgagtagcgtgactgcagcagatacagccgtgtattattgcgccaaagctccctacatgatgtacttcgactcttggggtcagggaacactcgttaccgtgtcatctgccagcacaaagggccccagcgtctttccgttagctcccagttcaaagtctactagtggtggtaccgcagctctgggctgtctggtcaaggactacttcccagaaccggtgactgtatcttggaatagcggggctcttactagcggagtgcacacttttcccgcagtccttcagtcctcaggattatacagtctcagcagtgttgttaccgtgcctagctccagtttgggcacgcaaacgtatatctgcaatgtcaaccataaaccttccaatacgaaagtggacaaacgagtggaaccaaagtcctgtgggggcgggggatccgaggtacgattgcagcaatcagggcccgacctcatcaaacctggggcatcagtcaagatgtcttgtaaggcatccggctatacctttaccggatacgttatgcactgggtcaaacagcggcctggtcagggacttgagtggatcggtttcattaatccatacaacgacgacattcagagcaatgagcggtttcgcgggaaagcgacactgacgagtgacaagagcagcactactgcctatatggagctgtctagcctgacctccgaggatagcgccgtctactattgcgcaagaggcgccggctacaacttcgatggggcttacagattcttcgatttctggggccaaggaaccaccctgacagtgtccagcggaggaggcgggtcaggaggaggagggtctggcggcggtggctctgacgtggtgatgactcagagccctctgtcattgcccgtgagccttggcgatcaggccagcatcagctgtaggtctagccagagactggtccactctaacggcaatacctatctccactggtatctgcagaaacccgggcaatccccaaaactgctgatctaccgcgtttctaaccgctttcctggcgtacccgacaggttttcagggtccggctcaggaacagactttaccctgaagataagtcgtgtagaggcggaggatctggggatctacttctgcagtcagagcacacatgtgccgtataccttcggaggcggtactaagctggaaattaagcggcatcaccaccatcaccat

SEQ ID NO: 47 - DNA, 642 bp, synthetic construct
  source 1..642: mol_type = other DNA; note = Nucleotide sequence encoding CD1a1001 VL
gacatccagatgacacagtctccatccagcttgtctgctagtgtcggagatagggtgactatcacctgtagagcctctcagtccatatcctcctatctgaactggtatcagcagaaaccaggcaaagcacccaagctcctgatctatgctgcctcaagcctgcagtcaggcgttccttctcggttttccggttcaggcagtggaaccgacttcaccctgacgattagcagccttcaacccgaagatttcgccacctactactgccagcagagctacagtacacctcccacttttgggcaagggacaaaggtggagattaagcgaacagtggctgctccttctgtgttcatctttccacccagcgacgaacagctgaagtctggaactgcctctgttgtgtgtctcctgaacaacttctatcccagagaagccaaggtacagtggaaagtggacaatgcgttgcagagtggcaactcccaggagagcgttactgagcaggatagcaaggacagtacctactccttgagctccacgctgacccttagcaaagccgattacgagaagcacaaggtctatgcgtgcgaagtcactcaccaaggcctgtcaagtccagtgaccaagtctttcaatcgtggggaatgc

SEQ ID NO: 48 - DNA, 1446 bp, synthetic construct
  source 1..1446: mol_type = other DNA; note = Nucleotide sequence encoding CD1a1003 VH
caggtacagttgcaggaatctggcgctggattgctgaagccatccgagactctgagcctgacatgtgccgtctatggtggctccttttccgggtattactggagctggattcggcaacctcctggcaaagggcttgagtggataggctacatctactattccggaagcaccaactacaatccctcactcaagagtagggtcaccatcagtgtggacacgtctaagaaccagttctccctgaagctgagtagcgtgactgcagcagatacagccgtgtattattgcgccaaagctccctacatgatgtacttcgactcttggggtcagggaacactcgttaccgtgtcatctgccagcacaaagggccccagcgtctttccgttagctcccagttcaaagtctactagtggtggtaccgcagctctgggctgtctggtcaaggactacttcccagaaccggtgactgtatcttggaatagcggggctcttactagcggagtgcacacttttcccgcagtccttcagtcctcaggattatacagtctcagcagtgttgttaccgtgcctagctccagtttgggcacgcaaacgtatatctgcaatgtcaaccataaaccttccaatacgaaagtggacaaacgagtggaaccaaagtcctgtgggggcgggggatcccaggttcagctcgtacagagtggagctgaagtcaagaaaccaggtgcatcagtcaaggtgtcctgcaaagcttcagggtataagtttacagggttcgtgatgcactgggtgagacaggctcctggacaaggcctggaatggatgggcttcatcaacccctacaatgacgacatccagtccaatgagcgatttcgtggtagggtgacgatgacacgggatacctccattagcactgcctatatggagctgtctcgcttgaggagtgacgatactgccgtttactactgtgccagaggtaacggctacaacttcgatggggcctatcggttcttcgacttttggggacaaggcaccatggtcacagtgtctagcggaggaggcgggtcaggaggaggagggtctggcggcggtggctctgacattgtgatgactcagtcacccctttctctgcccgttactcctggagaaccagccagcatatcctgccgttctagccagaggttggtgcactccaatgggaacacctatctgcactggtatctccagaaaccaggacagagtcctagactgctgatctaccgagtcagcaaccgctttccaggtgttcctgatcggttctcaggttctgggagtggcacagacttcacgctcaagatctccagggtcgaagctgaggatgtaggcgtgtactactgtagccagtccacacatgtgccctatacctttggacaaggcaccaaactggagattaagcatcaccaccatcaccat

SEQ ID NO: 49 - DNA, 2112 bp, synthetic construct
  source 1..2112: mol_type = other DNA; note = Nucleotide sequence encoding CD1a1004 VH
caggtacagttgcaggaatctggcgctggattgctgaagccatccgagactctgagcctgacatgtgccgtctatggtggctccttttccgggtattactggagctggattcggcaacctcctggcaaagggcttgagtggataggctacatctactattccggaagcaccaactacaatccctcactcaagagtagggtcaccatcagtgtggacacgtctaagaaccagttctccctgaagctgagtagcgtgactgcagcagatacagccgtgtattattgcgccaaagctccctacatgatgtacttcgactcttggggtcagggaacactcgttaccgtgtcatctgccagcacaaagggccccagcgtctttccgttagctcccagttcaaagtctactagtggtggtaccgcagctctgggctgtctggtcaaggactacttcccagaaccggtgactgtatcttggaatagcggggctcttactagcggagtgcacacttttcccgcagtccttcagtcctcaggattatacagtctcagcagtgttgttaccgtgcctagctccagtttgggcacgcaaacgtatatctgcaatgtcaaccataaaccttccaatacgaaagtggacaaacgagtggaaccaaagtcctgtgggggcgggggatccgaggtacgattgcagcaatcagggcccgacctcatcaaacctggggcatcagtcaagatgtcttgtaaggcatccggctatacctttaccggatacgttatgcactgggtcaaacagcggcctggtcagggacttgagtggatcggtttcattaatccatacaacgacgacattcagagcaatgagcggtttcgcgggaaagcgacactgacgagtgacaagagcagcactactgcctatatggagctgtctagcctgacctccgaggatagcgccgtctactattgcgcaagaggcgccggctacaacttcgatggggcttacagattcttcgatttctggggccaaggaaccaccctgacagtgtccagcggaggaggcgggtcaggaggaggagggtctggcggcggtggctctgacgtggtgatgactcagagccctctgtcattgcccgtgagccttggcgatcaggccagcatcagctgtaggtctagccagagactggtccactctaacggcaatacctatctccactggtatctgcagaaacccgggcaatccccaaaactgctgatctaccgcgtttctaaccgctttcctggcgtacccgacaggttttcagggtccggctcaggaacagactttaccctgaagataagtcgtgtagaggcggaggatctggggatctacttctgcagtcagagcacacatgtgccgtataccttcggaggcggtactaagctggaaattaagcgggacaagacccatacttgtcctccgtgtcctgcccctgaagcggccggaggtccatccgtcttcctgtttccccctaaacctaaggataccctgatgatctccaggacaccggaagtgacctgtgtcgttgttgacgtgagccatgaagatcccgaggtgaagttcaactggtatgtggatggagtggaggtacacaatgccaagacaaagccacgagaggagcagtacaactcaacataccgggttgtgtctgtgcttacagtgctccatcaagactggctgaacggcaaagagtacaagtgcaaagtttccaacaaagccttacctgctcccattgagaagaccatcagcaaggcaaaggggcaaccacgagaaccccaggtgtacacacttcctccatcccgggaagagatgacaaagaaccaggtgtcacttacatgcctcgtaaaagggttttacccatccgacatagccgttgagtgggagtctaatggccagcccgagaacaactacaagacaactccgccagtgctggattcggacgggtcttttttcctatacagtaagctgaccgtcgataaaagccggtggcaacagggcaacgtgttctcttgttccgtcatgcacgaagctcttcacaaccactacacccagaaatctctgagtttgagtcccggaaag

SEQ ID NO: 50 - DNA, 2109 bp, synthetic construct
  source 1..2109: mol_type = other DNA; note = Nucleotide sequence encoding CD1a1006 VH
caggtacagttgcaggaatctggcgctggattgctgaagccatccgagactctgagcctgacatgtgccgtctatggtggctccttttccgggtattactggagctggattcggcaacctcctggcaaagggcttgagtggataggctacatctactattccggaagcaccaactacaatccctcactcaagagtagggtcaccatcagtgtggacacgtctaagaaccagttctccctgaagctgagtagcgtgactgcagcagatacagccgtgtattattgcgccaaagctccctacatgatgtacttcgactcttggggtcagggaacactcgttaccgtgtcatctgccagcacaaagggccccagcgtctttccgttagctcccagttcaaagtctactagtggtggtaccgcagctctgggctgtctggtcaaggactacttcccagaaccggtgactgtatcttggaatagcggggctcttactagcggagtgcacacttttcccgcagtccttcagtcctcaggattatacagtctcagcagtgttgttaccgtgcctagctccagtttgggcacgcaaacgtatatctgcaatgtcaaccataaaccttccaatacgaaagtggacaaacgagtggaaccaaagtcctgtgggggcgggggatcccaggttcagctcgtacagagtggagctgaagtcaagaaaccaggtgcatcagtcaaggtgtcctgcaaagcttcagggtataagtttacagggttcgtgatgcactgggtgagacaggctcctggacaaggcctggaatggatgggcttcatcaacccctacaatgacgacatccagtccaatgagcgatttcgtggtagggtgacgatgacacgggatacctccattagcactgcctatatggagctgtctcgcttgaggagtgacgatactgccgtttactactgtgccagaggtaacggctacaacttcgatggggcctatcggttcttcgacttttggggacaaggcaccatggtcacagtgtctagcggaggaggcgggtcaggaggaggagggtctggcggcggtggctctgacattgtgatgactcagtcacccctttctctgcccgttactcctggagaaccagccagcatatcctgccgttctagccagaggttggtgcactccaatgggaacacctatctgcactggtatctccagaaaccaggacagagtcctagactgctgatctaccgagtcagcaaccgctttccaggtgttcctgatcggttctcaggttctgggagtggcacagacttcacgctcaagatctccagggtcgaagctgaggatgtaggcgtgtactactgtagccagtccacacatgtgccctatacctttggacaaggcaccaaactggagattaaggacaagacccatacttgtcctccgtgtcctgcccctgaagcggccggaggtccatccgtcttcctgtttccccctaaacctaaggataccctgatgatctccaggacaccggaagtgacctgtgtcgttgttgacgtgagccatgaagatcccgaggtgaagttcaactggtatgtggatggagtggaggtacacaatgccaagacaaagccacgagaggagcagtacaactcaacataccgggttgtgtctgtgcttacagtgctccatcaagactggctgaacggcaaagagtacaagtgcaaagtttccaacaaagccttacctgctcccattgagaagaccatcagcaaggcaaaggggcaaccacgagaaccccaggtgtacacacttcctccatcccgggaagagatgacaaagaaccaggtgtcacttacatgcctcgtaaaagggttttacccatccgacatagccgttgagtgggagtctaatggccagcccgagaacaactacaagacaactccgccagtgctggattcggacgggtcttttttcctatacagtaagctgaccgtcgataaaagccggtggcaacagggcaacgtgttctcttgttccgtcatgcacgaagctcttcacaaccactacacccagaaatctctgagtttgagtcccggaaag

SEQ ID NO: 51 - protein, 5 aa, synthetic construct
  source 1..5: note = G4S
GGGGS

SEQ ID NO: 52 - protein, 10 aa, synthetic construct
  source 1..10: note = (G4S)2
GGGGSGGGGS

SEQ ID NO: 53 - protein, 10 aa, synthetic construct
  source 1..10: note = (SG4)2
SGGGGSGGGG

SEQ ID NO: 54 - protein, 14 aa, synthetic construct
  source 1..14: note = (G4S)2G4
GGGGSGGGGSGGGG

SEQ ID NO: 55 - protein, 10 aa, synthetic construct
  source 1..10: note = GSPGSSSSGS
GSPGSSSSGS

SEQ ID NO: 56 - protein, 8 aa, synthetic construct
  source 1..8: note = (GS)4
GSGSGSGS

SEQ ID NO: 57 - protein, 8 aa, synthetic construct
  source 1..8: note = GSGSGNGS
GSGSGNGS

SEQ ID NO: 58 - protein, 8 aa, synthetic construct
  source 1..8: note = GGSGSGSG
GGSGSGSG

SEQ ID NO: 59 - protein, 6 aa, synthetic construct
  source 1..6: note = GGSGSG
GGSGSG

SEQ ID NO: 60 - protein, 4 aa, synthetic construct
  source 1..4: note = GGSG
GGSG

SEQ ID NO: 61 - protein, 8 aa, synthetic construct
  source 1..8: note = GGSGNGSG
GGSGNGSG

SEQ ID NO: 62 - protein, 8 aa, synthetic construct
  source 1..8: note = GGNGSGSG
GGNGSGSG

SEQ ID NO: 63 - protein, 6 aa, synthetic construct
  source 1..6: note = GGNGSG
GGNGSG

SEQ ID NO: 64 - protein, 15 aa, synthetic construct
  source 1..15: note = (G4S)3
GGGGSGGGGSGGGGS

SEQ ID NO: 65 - protein, 703 aa, synthetic construct; identical to SEQ ID NO: 33
  source 1..703: note = CD1a1006 VH

SEQ ID NO: 66 - protein, 699 aa, synthetic construct
  source 1..699: note = CCR91002 VH
QVQLKESGPGLVQPSQTLSLTCTVSGFSVASYDMHWVRLPPGKGLEWMGIIWANGNTHYNSGLKSRLSISRDTSKSQVFLKMNSLQTEDTAIYFCTRGGFAYWGQGTLVTVSSASTKGPSVFPLAPSSKSTSGGTAALGCLVKDYFPEPVTVSWNSGALTSGVHTFPAVLQSSGLYSLSSVVTVPSSSLGTQTYICNVNHKPSNTKVDKRVEPKSCGGGGSQVQLVQSGAEVKKPGASVKVSCKASGYTFTGYVMHWVRQAPGQGLEWMGFINPYNDDIQSNERFRGRVTMTRDTSISTAYMELSRLRSDDTAVYYCARGAGYNFDGAYRFFDFWGQGTMVTVSSGGGGSGGGGSGGGGSDIVMTQSPLSLPVTPGEPASISCRSSQRLVHSNGNTYLHWYLQKPGQSPRLLIYRVSNRFPGVPDRFSGSGSGTDFTLKISRVEAEDVGVYYCSQSTHVPYTFGQGTKLEIKDKTHTCPPCPAPEAAGGPSVFLFPPKPKDTLMISRTPEVTCVVVDVSHEDPEVKFNWYVDGVEVHNAKTKPREEQYNSTYRVVSVLTVLHQDWLNGKEYKCKVSNKALPAPIEKTISKAKGQPREPQVYTLPPSREEMTKNQVSLTCLVKGFYPSDIAVEWESNGQPENNYKTTPPVLDSDGSFFLYSKLTVDKSRWQQGNVFSCSVMHEALHNHYTQKSLSLSPGK

SEQ ID NO: 67 - protein, 218 aa, synthetic construct
  source 1..218: note = CCR91002 VL
DVVMTQTPVSLSVSLGGQVSISCRSSQSLVHNNGNTYLSWYLQKPGQSPQLLIYKVSNRFSGVSDRFSGSGSGTDFTLKISRVEPDDLGVYYCGQGTQYPTFGGGTKLELKRTVAAPSVFIFPPSDEQLKSGTASVVCLLNNFYPREAKVQWKVDNALQSGNSQESVTEQDSKDSTYSLSSTLTLSKADYEKHKVYACEVTHQGLSSPVTKSFNRGEC

SEQ ID NO: 68 - protein, 699 aa, synthetic construct
  source 1..699: note = CCR91004 VH
QVQLKESGPGLVQPSQTLSLTCTVSGFSVASYDMHWVRLPPGKGLEWMGIIWANGNTHYNSGLKSRLSISRDTSKSQVFLKMNSLQTEDTAIYFCTRGGFAYWGQGTLVTVSSASTKGPSVFPLAPSSKSTSGGTAALGCLVKDYFPEPVTVSWNSGALTSGVHTFPAVLQSSGLYSLSSVVTVPSSSLGTQTYICNVNHKPSNTKVDKRVEPKSCDKTHTCPPCPAPEAAGGPSVFLFPPKPKDTLMISRTPEVTCVVVDVSHEDPEVKFNWYVDGVEVHNAKTKPREEQYNSTYRVVSVLTVLHQDWLNGKEYKCKVSNKALPAPIEKTISKAKGQPREPQVYTLPPSREEMTKNQVSLTCLVKGFYPSDIAVEWESNGQPENNYKTTPPVLDSDGSFFLYSKLTVDKSRWQQGNVFSCSVMHEALHNHYTQKSLSLSPGKGGGGSQVQLVQSGAEVKKPGASVKVSCKASGYTFTGYVMHWVRQAPGQGLEWMGFINPYNDDIQSNERFRGRVTMTRDTSISTAYMELSRLRSDDTAVYYCARGAGYNFDGAYRFFDFWGQGTMVTVSSGGGGSGGGGSGGGGSDIVMTQSPLSLPVTPGEPASISCRSSQRLVHSNGNTYLHWYLQKPGQSPRLLIYRVSNRFPGVPDRFSGSGSGTDFTLKISRVEAEDVGVYYCSQSTHVPYTFGQGTKLEIK

SEQ ID NO: 69 - protein, 706 aa, synthetic construct
  source 1..706: note = CXCR41002 VH
EVQLVESGGGLVQPGRSLRLSCTASGFTFTDNYMSWVRQAPGKGLEWVGFIRNKANGYTTEYAASVKGRFTISRDNSKSIAYLQMNSLKTEDTAVYYCARDVGSNYFDYWGQGTLVTVSSASTKGPSVFPLAPSSKSTSGGTAALGCLVKDYFPEPVTVSWNSGALTSGVHTFPAVLQSSGLYSLSSVVTVPSSSLGTQTYICNVNHKPSNTKVDKRVEPKSCGGGGSQVQLVQSGAEVKKPGASVKVSCKASGYTFTGYVMHWVRQAPGQGLEWMGFINPYNDDIQSNERFRGRVTMTRDTSISTAYMELSRLRSDDTAVYYCARGAGYNFDGAYRFFDFWGQGTMVTVSSGGGGSGGGGSGGGGSDIVMTQSPLSLPVTPGEPASISCRSSQRLVHSNGNTYLHWYLQKPGQSPRLLIYRVSNRFPGVPDRFSGSGSGTDFTLKISRVEAEDVGVYYCSQSTHVPYTFGQGTKLEIKDKTHTCPPCPAPEAAGGPSVFLFPPKPKDTLMISRTPEVTCVVVDVSHEDPEVKFNWYVDGVEVHNAKTKPREEQYNSTYRVVSVLTVLHQDWLNGKEYKCKVSNKALPAPIEKTISKAKGQPREPQVYTLPPSREEMTKNQVSLTCLVKGFYPSDIAVEWESNGQPENNYKTTPPVLDSDGSFFLYSKLTVDKSRWQQGNVFSCSVMHEALHNHYTQKSLSLSPGK

SEQ ID NO: 70 - protein, 219 aa, synthetic construct
  source 1..219: note = CXCR41002 VL
DIVMTQSPSSLAVSLGERATMSCKSSQSLFNSRTRKNYLAWYQQKPGQSPKLLIYWASARDSGVPARFTGSGSETYFTLTISRVQAEDLAVYYCMQSFNLRTFGQGTKVEIKRTVAAPSVFIFPPSDEQLKSGTASVVCLLNNFYPREAKVQWKVDNALQSGNSQESVTEQDSKDSTYSLSSTLTLSKADYEKHKVYACEVTHQGLSSPVTKSFNRGEC

SEQ ID NO: 71 - protein, 706 aa, synthetic construct
  source 1..706: note = CXCR41004 VH
EVQLVESGGGLVQPGRSLRLSCTASGFTFTDNYMSWVRQAPGKGLEWVGFIRNKANGYTTEYAASVKGRFTISRDNSKSIAYLQMNSLKTEDTAVYYCARDVGSNYFDYWGQGTLVTVSSASTKGPSVFPLAPSSKSTSGGTAALGCLVKDYFPEPVTVSWNSGALTSGVHTFPAVLQSSGLYSLSSVVTVPSSSLGTQTYICNVNHKPSNTKVDKRVEPKSCDKTHTCPPCPAPEAAGGPSVFLFPPKPKDTLMISRTPEVTCVVVDVSHEDPEVKFNWYVDGVEVHNAKTKPREEQYNSTYRVVSVLTVLHQDWLNGKEYKCKVSNKALPAPIEKTISKAKGQPREPQVYTLPPSREEMTKNQVSLTCLVKGFYPSDIAVEWESNGQPENNYKTTPPVLDSDGSFFLYSKLTVDKSRWQQGNVFSCSVMHEALHNHYTQKSLSLSPGKGGGGSQVQLVQSGAEVKKPGASVKVSCKASGYTFTGYVMHWVRQAPGQGLEWMGFINPYNDDIQSNERFRGRVTMTRDTSISTAYMELSRLRSDDTAVYYCARGAGYNFDGAYRFFDFWGQGTMVTVSSGGGGSGGGGSGGGGSDIVMTQSPLSLPVTPGEPASISCRSSQRLVHSNGNTYLHWYLQKPGQSPRLLIYRVSNRFPGVPDRFSGSGSGTDFTLKISRVEAEDVGVYYCSQSTHVPYTFGQGTKLEIK

SEQ ID NO: 72 - protein, 705 aa, synthetic construct
  source 1..705: note = TIG2001 VH
EVQLVQSGAEVKKPGSSVKVSCKASGYTFSSYVMHWVRQAPGQGLEWIGYIDPYNDGAKYAQKFQGRVTLTSDKSTSTAYMELSSLRSEDTAVYYCARGGPYGWYFDVWGQGTTVTVSSASTKGPSVFPLAPGGKSTSGGTAALGCLVKDYFPEPVTVSWNSGALTSGVHTFPAVLQSSGLYSLSSVVTVPSSSLGTQTYICNVNHKPSNTKVDKKVEPKSCGGGGSQVQLVQSGAEVKKPGASVKVSCKASGYTFTGYVMHWVRQAPGQGLEWMGFINPYNDDIQSNERFRGRVTMTRDTSISTAYMELSRLRSDDTAVYYCARGAGYNFDGAYRFFDFWGQGTMVTVSSGGGGSGGGGSGGGGSDIVMTQSPLSLPVTPGEPASISCRSSQRLVHSNGNTYLHWYLQKPGQSPRLLIYRVSNRFPGVPDRFSGSGSGTDFTLKISRVEAEDVGVYYCSQSTHVPYTFGQGTKLEIKDKTHTCPPCPAPEAAGGPSVFLFPPKPKDTLMISRTPEVTCVVVDVSHEDPEVKFNWYVDGVEVHNAKTKPREEQYNSTYRVVSVLTVLHQDWLNGKEYKCKVSNKALPAPIEKTISKAKGQPREPQVYTLPPSREEMTKNQVSLTCLVKGFYPSDIAVEWESNGQPENNYKTTPPVLDSDGSFFLYSKLTVDKSRWQQGNVFSCSVMHEALHNHYTQKSLSLSPGK

SEQ ID NO: 73 - protein, 214 aa, synthetic construct
  source 1..214: note = TIG2001 VL
DIQMTQSPSSLSASVGDRVTITCRASEHIYSYLSWYQQKPGKVPKLLIYNAKTLAEGVPSRFSGSGSGTDFTLTISSLQPEDVATYYCQHHFGSPLTFGQGTRLEIKRTVAAPSVFIFPPSDEQLKSGTASVVCLLNNFYPREAKVQWKVDNALQSGNSQESVTEQDSKDSTYSLSSTLTLSKADYEKHKVYACEVTHQGLSSPVTKSFNRGEC

SEQ ID NO: 74 - protein, 705 aa, synthetic construct
  source 1..705: note = TIG2002 VH
EVQLVQSGAEVKKPGSSVKVSCKASGYTFSSYVMHWVRQAPGQGLEWIGYIDPYNDGAKYAQKFQGRVTLTSDKSTSTAYMELSSLRSEDTAVYYCARGGPYGWYFDVWGQGTTVTVSSASTKGPSVFPLAPGGKSTSGGTAALGCLVKDYFPEPVTVSWNSGALTSGVHTFPAVLQSSGLYSLSSVVTVPSSSLGTQTYICNVNHKPSNTKVDKKVEPKSCDKTHTCPPCPAPEAAGGPSVFLFPPKPKDTLMISRTPEVTCVVVDVSHEDPEVKFNWYVDGVEVHNAKTKPREEQYNSTYRVVSVLTVLHQDWLNGKEYKCKVSNKALPAPIEKTISKAKGQPREPQVYTLPPSREEMTKNQVSLTCLVKGFYPSDIAVEWESNGQPENNYKTTPPVLDSDGSFFLYSKLTVDKSRWQQGNVFSCSVMHEALHNHYTQKSLSLSPGKGGGGSQVQLVQSGAEVKKPGASVKVSCKASGYTFTGYVMHWVRQAPGQGLEWMGFINPYNDDIQSNERFRGRVTMTRDTSISTAYMELSRLRSDDTAVYYCARGAGYNFDGAYRFFDFWGQGTMVTVSSGGGGSGGGGSGGGGSDIVMTQSPLSLPVTPGEPASISCRSSQRLVHSNGNTYLHWYLQKPGQSPRLLIYRVSNRFPGVPDRFSGSGSGTDFTLKISRVEAEDVGVYYCSQSTHVPYTFGQGTKLEIK

SEQ ID NO: 75 - protein, 706 aa, synthetic construct
  source 1..706: note = CCR81001 VH
EVQLVESGGGLVQPGGSLKLSCAASGFIFSNAVMYWVRQASGKGLEWVARIKTKFNNYATYYADAVKGRFTISRDDSKNMVYLQMNSLKTEDTAVYYCTAGDRNKPFAYWGQGTLVTVSSASTKGPSVFPLAPSSKSTSGGTAALGCLVKDYFPEPVTVSWNSGALTSGVHTFPAVLQSSGLYSLSSVVTVPSSSLGTQTYICNVNHKPSNTKVDKKVEPKSCGGGGSQVQLVQSGAEVKKPGASVKVSCKASGYTFTGYVMHWVRQAPGQGLEWMGFINPYNDDIQSNERFRGRVTMTRDTSISTAYMELSRLRSDDTAVYYCARGAGYNFDGAYRFFDFWGQGTMVTVSSGGGGSGGGGSGGGGSDIVMTQSPLSLPVTPGEPASISCRSSQRLVHSNGNTYLHWYLQKPGQSPRLLIYRVSNRFPGVPDRFSGSGSGTDFTLKISRVEAEDVGVYYCSQSTHVPYTFGQGTKLEIKDKTHTCPPCPAPEAAGGPSVFLFPPKPKDTLMISRTPEVTCVVVDVSHEDPEVKFNWYVDGVEVHNAKTKPREEQYNSTYRVVSVLTVLHQDWLNGKEYKCKVSNKALPAPIEKTISKAKGQPREPQVYTLPPSREEMTKNQVSLTCLVKGFYPSDIAVEWESNGQPENNYKTTPPVLDSDGSFFLYSKLTVDKSRWQQGNVFSCSVMHEALHNHYTQKSLSLSPGK

SEQ ID NO: 76 - protein, 214 aa, synthetic construct
  source 1..214: note = CCR81001 VL
ETVVTQSPATLSLSPGERATLSCRASTSVITLLHWFQQKPGQAPRLLIHGASNLESRVPARFSGSGSGTDFTLTISSLEPEDFATYFCQQSWNDPYTFGQGTKLEIKRTVAAPSVFIFPPSDEQLKSGTASVVCLLNNFYPREAKVQWKVDNALQSGNSQESVTEQDSKDSTYSLSSTLTLSKADYEKHKVYACEVTHQGLSSPVTKSFNRGEC

SEQ ID NO: 77 - protein, 706 aa, synthetic construct
  source 1..706: note = CCR81002 VH
EVQLVESGGGLVQPGGSLKLSCAASGFIFSNAVMYWVRQASGKGLEWVARIKTKFNNYATYYADAVKGRFTISRDDSKNMVYLQMNSLKTEDTAVYYCTAGDRNKPFAYWGQGTLVTVSSASTKGPSVFPLAPSSKSTSGGTAALGCLVKDYFPEPVTVSWNSGALTSGVHTFPAVLQSSGLYSLSSVVTVPSSSLGTQTYICNVNHKPSNTKVDKKVEPKSCDKTHTCPPCPAPEAAGGPSVFLFPPKPKDTLMISRTPEVTCVVVDVSHEDPEVKFNWYVDGVEVHNAKTKPREEQYNSTYRVVSVLTVLHQDWLNGKEYKCKVSNKALPAPIEKTISKAKGQPREPQVYTLPPSREEMTKNQVSLTCLVKGFYPSDIAVEWESNGQPENNYKTTPPVLDSDGSFFLYSKLTVDKSRWQQGNVFSCSVMHEALHNHYTQKSLSLSPGKGGGGSQVQLVQSGAEVKKPGASVKVSCKASGYTFTGYVMHWVRQAPGQGLEWMGFINPYNDDIQSNERFRGRVTMTRDTSISTAYMELSRLRSDDTAVYYCARGAGYNFDGAYRFFDFWGQGTMVTVSSGGGGSGGGGSGGGGSDIVMTQSPLSLPVTPGEPASISCRSSQRLVHSNGNTYLHWYLQKPGQSPRLLIYRVSNRFPGVPDRFSGSGSGTDFTLKISRVEAEDVGVYYCSQSTHVPYTFGQGTKLEIK

SEQ ID NO: 78 - protein, 482 aa, synthetic construct
  source 1..482: note = CD301001 VH
QIQLQQSGPEVVKPGASVKISCKASGYTFTDYYITWVKQKPGQGLEWIGWIYPGSGNTKYNEKFKGKATLTVDTSSSTAFMQLSSLTSEDTAVYFCANYGNYWFAYWGQGTQVTVSAASTKGPSVFPLAPSSKSTSGGTAALGCLVKDYFPEPVTVSWNSGALTSGVHTFPAVLQSSGLYSLSSVVTVPSSSLGTQTYICNVNHKPSNTKVDKRVEPKSCGGGGSQVQLVQSGAEVKKPGASVKVSCKASGYTFTGYVMHWVRQAPGQGLEWMGFINPYNDDIQSNERFRGRVTMTRDTSISTAYMELSRLRSDDTAVYYCARGAGYNFDGAYRFFDFWGQGTMVTVSSGGGGSGGGGSGGGGSDIVMTQSPLSLPVTPGEPASISCRSSQRLVHSNGNTYLHWYLQKPGQSPRLLIYRVSNRFPGVPDRFSGSGSGTDFTLKISRVEAEDVGVYYCSQSTHVPYTFGQGTKLEIKHHHHHH

SEQ ID NO: 79 - protein, 218 aa, synthetic construct
  source 1..218: note = CD301001 VL
DIVLTQSPASLAVSLGQRATISCKASQSVDFDGDSYMNWYQQKPGQPPKVLIYAASNLESGIPARFSGSGSGTDFTLNIHPVEEEDAATYYCQQSNEDPWTFGGGTKLEIKRTVAAPSVFIFPPSDEQLKSGTASVVCLLNNFYPREAKVQWKVDNALQSGNSQESVTEQDSKDSTYSLSSTLTLSKADYEKHKVYACEVTHQGLSSPVTKSFNRGEC

SEQ ID NO: 80 - protein, 703 aa, synthetic construct
  source 1..703: note = CD301003 VH
QIQLQQSGPEVVKPGASVKISCKASGYTFTDYYITWVKQKPGQGLEWIGWIYPGSGNTKYNEKFKGKATLTVDTSSSTAFMQLSSLTSEDTAVYFCANYGNYWFAYWGQGTQVTVSAASTKGPSVFPLAPSSKSTSGGTAALGCLVKDYFPEPVTVSWNSGALTSGVHTFPAVLQSSGLYSLSSVVTVPSSSLGTQTYICNVNHKPSNTKVDKRVEPKSCGGGGSQVQLVQSGAEVKKPGASVKVSCKASGYTFTGYVMHWVRQAPGQGLEWMGFINPYNDDIQSNERFRGRVTMTRDTSISTAYMELSRLRSDDTAVYYCARGAGYNFDGAYRFFDFWGQGTMVTVSSGGGGSGGGGSGGGGSDIVMTQSPLSLPVTPGEPASISCRSSQRLVHSNGNTYLHWYLQKPGQSPRLLIYRVSNRFPGVPDRFSGSGSGTDFTLKISRVEAEDVGVYYCSQSTHVPYTFGQGTKLEIKDKTHTCPPCPAPEAAGGPSVFLFPPKPKDTLMISRTPEVTCVVVDVSHEDPEVKFNWYVDGVEVHNAKTKPREEQYNSTYRVVSVLTVLHQDWLNGKEYKCKVSNKALPAPIEKTISKAKGQPREPQVYTLPPSREEMTKNQVSLTCLVKGFYPSDIAVEWESNGQPENNYKTTPPVLDSDGSFFLYSKLTVDKSRWQQGNVFSCSVMHEALHNHYTQKSLSLSPGK

SEQ ID NO: 81 - protein, 704 aa, synthetic construct
  source 1..704: note = CD40L1007 VH
QVQLVQSGAEVQKPGSSVKVSCKASGGTFSNFAFNWVRQVPGQGLEWMGRILPSLDIASYAQKFQDRVTITADKSTSTAYMELSSLRSEDTAMYYCAREVDGGGFDYWGQGTLVTVSSASTKGPSVFPLAPSSKSTSGGTAALGCLVKDYFPEPVTVSWNSGALTSGVHTFPAVLQSSGLYSLSSVVTVPSSSLGTQTYICNVNHKPSNTKVDKRVEPKSCDKTHTCPPCPAPEAAGGPSVFLFPPKPKDTLMISRTPEVTCVVVDVSHEDPEVKFNWYVDGVEVHNAKTKPREEQYNSTYRVVSVLTVLHQDWLNGKEYKCKVSNKALPAPIEKTISKAKGQPREPQVYTLPPSREEMTKNQVSLTCLVKGFYPSDIAVEWESNGQPENNYKTTPPVLDSDGSFFLYSKLTVDKSRWQQGNVFSCSVMHEALHNHYTQKSLSLSPGKGGGGSQVQLVQSGAEVKKPGASVKVSCKASGYTFTGYVMHWVRQAPGQGLEWMGFINPYNDDIQSNERFRGRVTMTRDTSISTAYMELSRLRSDDTAVYYCARGAGYNFDGAYRFFDFWGQGTMVTVSSGGGGSGGGGSGGGGSDIVMTQSPLSLPVTPGEPASISCRSSQRLVHSNGNTYLHWYLQKPGQSPRLLIYRVSNRFPGVPDRFSGSGSGTDFTLKISRVEAEDVGVYYCSQSTHVPYTFGQGTKLEIK

SEQ ID NO: 82 - protein, 214 aa, synthetic construct
  source 1..214: note = CD40L1007 VL
DIQMTQSPSSLSASVGDRVTITCRASQGISSWLAWYQQKPEKAPKSLIYAASSLQSGVPSRFSGSGSGTDFTLTISSLQPEDFATYYCQQYNSYPFTFGGGTKVEIKRTVAAPSVFIFPPSDEQLKSGTASVVCLLNNFYPREAKVQWKVDNALQSGNSQESVTEQDSKDSTYSLSSTLTLSKADYEKHKVYACEVTHQGLSSPVTKSFNRGEC

SEQ ID NO: 83 - protein, 704 aa, synthetic construct
  source 1..704: note = CD40L1008 VH
QVQLVQSGAEVQKPGSSVKVSCKASGGTFSNFAFNWVRQVPGQGLEWMGRILPSLDIASYAQKFQDRVTITADKSTSTAYMELSSLRSEDTAMYYCAREVDGGGFDYWGQGTLVTVSSASTKGPSVFPLAPSSKSTSGGTAALGCLVKDYFPEPVTVSWNSGALTSGVHTFPAVLQSSGLYSLSSVVTVPSSSLGTQTYICNVNHKPSNTKVDKRVEPKSCGGGGSQVQLVQSGAEVKKPGASVKVSCKASGYTFTGYVMHWVRQAPGQGLEWMGFINPYNDDIQSNERFRGRVTMTRDTSISTAYMELSRLRSDDTAVYYCARGAGYNFDGAYRFFDFWGQGTMVTVSSGGGGSGGGGSGGGGSDIVMTQSPLSLPVTPGEPASISCRSSQRLVHSNGNTYLHWYLQKPGQSPRLLIYRVSNRFPGVPDRFSGSGSGTDFTLKISRVEAEDVGVYYCSQSTHVPYTFGQGTKLEIKDKTHTCPPCPAPEAAGGPSVFLFPPKPKDTLMISRTPEVTCVVVDVSHEDPEVKFNWYVDGVEVHNAKTKPREEQYNSTYRVVSVLTVLHQDWLNGKEYKCKVSNKALPAPIEKTISKAKGQPREPQVYTLPPSREEMTKNQVSLTCLVKGFYPSDIAVEWESNGQPENNYKTTPPVLDSDGSFFLYSKLTVDKSRWQQGNVFSCSVMHEALHNHYTQKSLSLSPGK

SEQ ID NO: 84 - protein, 450 aa, synthetic construct
  source 1..450: note = TRBV50001 VH
QVQLKESGPGLVAPSQSLSITCTVSGFSLTAYGVNWVRQPPGKGLEWLGMIWGDGNTDYNSALKSRLSISKDNSKSQVFLKMNSLQTDDTARYYCARDRVTATLYAMDYWGQGTSVTVSSASTKGPSVFPLAPSSKSTSGGTAALGCLVKDYFPEPVTVSWNSGALTSGVHTFPAVLQSSGLYSLSSVVTVPSSSLGTQTYICNVNHKPSNTKVDKRVEPKSCDKTHTCPPCPAPEAAGGPSVFLFPPKPKDTLMISRTPEVTCVVVDVSHEDPEVKFNWYVDGVEVHNAKTKPREEQYNSTYRVVSVLTVLHQDWLNGKEYKCKVSNKALPAPIEKTISKAKGQPREPQVYTLPPSREEMTKNQVSLTCLVKGFYPSDIAVEWESNGQPENNYKTTPPVLDSDGSFLLYSKLTVDKSRWQQGNVFSCSVMHEALHNHYTQKSLSLSPGK

SEQ ID NO: 85 - protein, 214 aa, synthetic construct
  source 1..214: note = TRBV50001 VL
DIQMTQTTSSLSASLGDRVTITCSASQGISNYLNWYQQKPDGTVKLLIYYTSSLHSGVPSRFSGSGSGTDYSLTISNLEPEDIATYYCQQYSKLPRTFGGGTKVEIKRTVAAPSVFIFPPSDEQLKSGTASVVCLLNNFYPREAKVQWKVDNALQSGNSQESVTEQDSKDSTYSLSSTLTLSKADYEKHKVYACEVTHQGLSSPVTKSFNRGEC

SEQ ID NO: 86 - protein, 694 aa, synthetic construct
  source 1..694: note = TRBV50004 VH
QVQLQESGAGLLKPSETLSLTCAVYGGSFSGYYWSWIRQPPGKGLEWIGYIYYSGSTNYNPSLKSRVTISVDTSKNQFSLKLSSVTAADTAVYYCAKAPYMMYFDSWGQGTLVTVSSASTKGPSVFPLAPSSKSTSGGTAALGCLVKDYFPEPVTVSWNSGALTSGVHTFPAVLQSSGLYSLSSVVTVPSSSLGTQTYICNVNHKPSNTKVDKRVEPKSCGGGGSQVQLKESGPGLVAPSQSLSITCTVSGFSLTAYGVNWVRQPPGKGLEWLGMIWGDGNTDYNSALKSRLSISKDNSKSQVFLKMNSLQTDDTARYYCARDRVTATLYAMDYWGQGTSVTVSSGGGGSGGGGSGGGGSDIQMTQTTSSLSASLGDRVTITCSASQGISNYLNWYQQKPDGTVKLLIYYTSSLHSGVPSRFSGSGSGTDYSLTISNLEPEDIATYYCQQYSKLPRTFGGGTKVEIKDKTHTCPPCPAPEAAGGPSVFLFPPKPKDTLMISRTPEVTCVVVDVSHEDPEVKFNWYVDGVEVHNAKTKPREEQYNSTYRVVSVLTVLHQDWLNGKEYKCKVSNKALPAPIEKTISKAKGQPREPQVYTLPPSREEMTKNQVSLTCLVKGFYPSDIAVEWESNGQPENNYKTTPPVLDSDGSFFLYSKLTVDKSRWQQGNVFSCSVMHEALHNHYTQKSLSLSPGK

SEQ ID NO: 87 - protein, 703 aa, synthetic construct
  source 1..703: note = CD1a1005 VH
QVQLQESGAGLLKPSETLSLTCAVYGGSFSGYYWSWIRQPPGKGLEWIGYIYYSGSTNYNPSLKSRVTISVDTSKNQFSLKLSSVTAADTAVYYCAKAPYMMYFDSWGQGTLVTVSSASTKGPSVFPLAPSSKSTSGGTAALGCLVKDYFPEPVTVSWNSGALTSGVHTFPAVLQSSGLYSLSSVVTVPSSSLGTQTYICNVNHKPSNTKVDKRVEPKSCGGGGSQVQLVQSGAEVKKPGASVKVSCKASGYTFTGYVMHWVRQAPGQGLEWMGFINPYNDDIQSNERFRGRVTMTRDTSISTAYMELSRLRSDDTAVYYCARGAGYNFDGAYRFFDFWGQGTMVTVSSGGGGSGGGGSGGGGSDIVMTQSPLSLPVTPGEPASISCRSSQRLVHSNGNTYLHWYLQKPGQSPRLLIYRVSNRFPGVPDRFSGSGSGTDFTLKISRVEAEDVGVYYCSQSTHVPYTFGQGTKLEIKDKTHTCPPCPAPEAAGGPSVFLFPPKPKDTLMISRTPEVTCVVVDVSHEDPEVKFNWYVDGVEVHNAKTKPREEQYNSTYRVVSVLTVLHQDWLNGKEYKCKVSNKALPAPIEKTISKAKGQPREPQVYTLPPSREEMTKNQVSLTCLVKGFYPSDIAVEWESNGQPENNYKTTPPVLDSDGSFFLYSKLTVDKSRWQQGNVFSCSVMHEALHNHYTQKSLSLSPGK

SEQ ID NO: 88 - protein, 696 aa, synthetic construct
  source 1..696: note = CD1a1016 VH
QVQLQESGAGLLKPSETLSLTCAVYGGSFSGYYWSWIRQPPGKGLEWIGYIYYSGSTNYNPSLKSRVTISVDTSKNQFSLKLSSVTAADTAVYYCAKAPYMMYFDSWGQGTLVTVSSASTKGPSVFPLAPSSKSTSGGTAALGCLVKDYFPEPVTVSWNSGALTSGVHTFPAVLQSSGLYSLSSVVTVPSSSLGTQTYICNVNHKPSNTKVDKRVEPKSCGGGGSEVQLVESGGGLVQPGGSLRLSCAASGYSFTGYTMNWVRQAPGKGLEWVALINPYKGVSTYNQKFKDRFTISVDKSKNTAYLQMNSLRAEDTAVYYCARSGYYGDSDWYFDVWGQGTLVTVSSGGGGSGGGGSGGGGSDIQMTQSPSSLSASVGDRVTITCRASQDIRNYLNWYQQKPGKAPKLLIYYTSRLESGVPSRFSGSGSGTDYTLTISSLQPEDFATYYCQQGNTLPWTFGQGTKVEIKDKTHTCPPCPAPEAAGGPSVFLFPPKPKDTLMISRTPEVTCVVVDVSHEDPEVKFNWYVDGVEVHNAKTKPREEQYNSTYRVVSVLTVLHQDWLNGKEYKCKVSNKALPAPIEKTISKAKGQPREPQVYTLPPSREEMTKNQVSLTCLVKGFYPSDIAVEWESNGQPENNYKTTPPVLDSDGSFFLYSKLTVDKSRWQQGNVFSCSVMHEALHNHYTQKSLSLSPGK

SEQ ID NO: 89 - protein, 5 aa, synthetic construct
  source 1..5: note = TIGIT CDRH1
SYVMH

SEQ ID NO: 90 - protein, 17 aa, synthetic construct
  source 1..17: note = TIGIT CDRH2
YIDPYNDGAKYAQKFQG

SEQ ID NO: 91 - protein, 10 aa, synthetic construct
  source 1..10: note = TIGIT CDRH3
GGPYGWYFDV

SEQ ID NO: 92 - protein, 11 aa, synthetic construct
  source 1..11: note = TIGIT CDRL1
RASEHIYSYLS

SEQ ID NO: 93 - protein, 7 aa, synthetic construct
  source 1..7: note = TIGIT CDRL2
NAKTLAE

SEQ ID NO: 94 - protein, 9 aa, synthetic construct
  source 1..9: note = TIGIT CDRL3
QHHFGSPLT

SEQ ID NO: 95 - protein, 5 aa, synthetic construct
  source 1..5: note = CCR8 CDRH1
NAVMY

SEQ ID NO: 96 - protein, 19 aa, synthetic construct
  source 1..19: note = CCR8 CDRH2
RIKTKFNNYATYYADAVKG

SEQ ID NO: 97 - protein, 9 aa, synthetic construct
  source 1..9: note = CCR8 CDRH3
GDRNKPFAY

SEQ ID NO: 98 - protein, 11 aa, synthetic construct
  source 1..11: note = CCR8 CDRL1
RASTSVITLLH

SEQ ID NO: 99 - protein, 7 aa, synthetic construct
  source 1..7: note = CCR8 CDRL2
GASNLES

SEQ ID NO: 100 - protein, 9 aa, synthetic construct
  source 1..9: note = CCR8 CDRL3
QQSWNDPYT

SEQ ID NO: 101 - protein, 5 aa, synthetic construct
  source 1..5: note = CCR9 CDRH1
SYDMH

SEQ ID NO: 102 - protein, 16 aa, synthetic construct
  source 1..16: note = CCR9 CDRH2
IIWANGNTHYNSGLKS

SEQ ID NO: 103 - protein, 5 aa, synthetic construct
  source 1..5: note = CCR9 CDRH3
GGFAY

SEQ ID NO: 104 - protein, 16 aa, synthetic construct
  source 1..16: note = CCR9 CDRL1
RSSQSLVHNNGNTYLS

SEQ ID NO: 105 - protein, 7 aa, synthetic construct
  source 1..7: note = CCR9 CDRL2
KVSNRFS

SEQ ID NO: 106 - protein, 8 aa, synthetic construct
  source 1..8: note = CCR9 CDRL3
GQGTQYPT

SEQ ID NO: 107 - protein, 5 aa, synthetic construct
  source 1..5: note = CXCR4 CDRH1
DNYMS

SEQ ID NO: 108 - protein, 19 aa, synthetic construct
  source 1..19: note = CXCR4 CDRH2
FIRNKANGYTTEYAASVKG

SEQ ID NO: 109 - protein, 9 aa, synthetic construct
  source 1..9: note = CXCR4 CDRH3
DVGSNYFDY

SEQ ID NO: 110 - protein, 17 aa, synthetic construct
  source 1..17: note = CXCR4 CDRL1
KSSQSLFNSRTRKNYLA

SEQ ID NO: 111 - protein, 7 aa, synthetic construct
  source 1..7: note = CXCR4 CDRL2
WASARDS

SEQ ID NO: 112 - protein, 8 aa, synthetic construct
  source 1..8: note = CXCR4 CDRL3
MQSFNLRT

SEQ ID NO: 113 - protein, 5 aa, synthetic construct
  source 1..5: note = CD30 CDRH1
DYYIT

SEQ ID NO: 114 - protein, 17 aa, synthetic construct
  source 1..17: note = CD30 CDRH2
WIYPGSGNTKYNEKFKG

SEQ ID NO: 115 - protein, 8 aa, synthetic construct
  source 1..8: note = CD30 CDRH3
YGNYWFAY

SEQ ID NO: 116 - protein, 15 aa, synthetic construct
  source 1..15: note = CD30 CDRL1
KASQSVDFDGDSYMN

SEQ ID NO: 117 - protein, 7 aa, synthetic construct
  source 1..7: note = CD30 CDRL2
AASNLES

SEQ ID NO: 118 - protein, 9 aa, synthetic construct
  source 1..9: note = CD30 CDRL3
QQSNEDPWT

SEQ ID NO: 119 - protein, 5 aa, synthetic construct
  source 1..5: note = CD40L CDRH1
NFAFN

SEQ ID NO: 120 - protein, 17 aa, synthetic construct
  source 1..17: note = CD40L CDRH2
RILPSLDIASYAQKFQD

SEQ ID NO: 121 - protein, 9 aa, synthetic construct
  source 1..9: note = CD40L CDRH3
EVDGGGFDY

SEQ ID NO: 122 - protein, 11 aa, synthetic construct
  source 1..11: note = CD40L CDRL1
RASQGISSWLA

SEQ ID NO: 123 - protein, 7 aa, synthetic construct
  source 1..7: note = CD40L CDRL2
AASSLQS

SEQ ID NO: 124 - protein, 9 aa, synthetic construct
  source 1..9: note = CD40L CDRL3
QQYNSYPFT

SEQ ID NO: 125 - protein, 5 aa, synthetic construct
  source 1..5: note = TRBV5 CDRH1
AYGVN

SEQ ID NO: 126 - protein, 16 aa, synthetic construct
  source 1..16: note = TRBV5 CDRH2
MIWGDGNTDYNSALKS

SEQ ID NO: 127 - protein, 12 aa, synthetic construct
  source 1..12: note = TRBV5 CDRH3
DRVTATLYAMDY

SEQ ID NO: 128 - protein, 11 aa, synthetic construct
  source 1..11: note = TRBV5 CDRL1
SASQGISNYLN

SEQ ID NO: 129 - protein, 7 aa, synthetic construct
  source 1..7: note = TRBV5 CDRL2
YTSSLHS

SEQ ID NO: 130 - protein, 9 aa, synthetic construct
  source 1..9: note = TRBV5 CDRL3
QQYSKLPRT

SEQ ID NO: 131 - protein, 184 aa, synthetic construct
  source 1..184: note = anti-CCR9 antibody VH
QVQLKESGPGLVQPSQTLSLTCTVSGFSVASYDMHWVRLPPGKGLEWMGIIWANGNTHYNSGLKSRLSISRQVQLKESGPGLVQPSQTLSLTCTVSGFSVASYDMHWVRLPPGKGLEWMGIIWANGNTHYNSGLKSRLSISRDTSKSQVFLKMNSLQTEDTAIYFCTRGGFAYWGQGTLVTVSS

SEQ ID NO: 132 - protein, 111 aa, synthetic construct
  source 1..111: note = anti-CCR9 antibody VL
DVVMTQTPVSLSVSLGGQVSISCRSSQSLVHNNGNTYLSWYLQKPGQSPQLLIYKVSNRFSGVSDRFSGSGSGTDFTLKISRVEPDDLGVYYCGQGTQYPTFGGGTKLELK

SEQ ID NO: 133 - protein, 120 aa, synthetic construct
  source 1..120: note = anti-CXCR4 antibody VH
EVQLVESGGGLVQPGRSLRLSCTASGFTFTDNYMSWVRQAPGKGLEWVGFIRNKANGYTTEYAASVKGRFTISRDNSKSIAYLQMNSLKTEDTAVYYCARDVGSNYFDYWGQGTLVTVSS

SEQ ID NO: 134 - protein, 112 aa, synthetic construct
  source 1..112: note = anti-CXCR4 antibody VL
DIVMTQSPSSLAVSLGERATMSCKSSQSLFNSRTRKNYLAWYQQKPGQSPKLLIYWASARDSGVPARFTGSGSETYFTLTISRVQAEDLAVYYCMQSFNLRTFGQGTKVEIK

SEQ ID NO: 135 - protein, 119 aa, synthetic construct
  source 1..119: note = anti-TIGIT antibody VH
EVQLVQSGAEVKKPGSSVKVSCKASGYTFSSYVMHWVRQAPGQGLEWIGYIDPYNDGAKYAQKFQGRVTLTSDKSTSTAYMELSSLRSEDTAVYYCARGGPYGWYFDVWGQGTTVTVSS

SEQ ID NO: 136 - protein, 107 aa, synthetic construct
  source 1..107: note = anti-TIGIT antibody VL
DIQMTQSPSSLSASVGDRVTITCRASEHIYSYLSWYQQKPGKVPKLLIYNAKTLAEGVPSRFSGSGSGTDFTLTISSLQPEDVATYYCQHHFGSPLTFGQGTRLEIK

SEQ ID NO: 137 - protein, 120 aa, synthetic construct
  source 1..120: note = anti-CCR8 antibody VH
EVQLVESGGGLVQPGGSLKLSCAASGFIFSNAVMYWVRQASGKGLEWVARIKTKFNNYATYYADAVKGRFTISRDDSKNMVYLQMNSLKTEDTAVYYCTAGDRNKPFAYWGQGTLVTVSS

SEQ ID NO: 138 - protein, 107 aa, synthetic construct
  source 1..107: note = anti-CCR8 antibody VL
ETVVTQSPATLSLSPGERATLSCRASTSVITLLHWFQQKPGQAPRLLIHGASNLESRVPARFSGSGSGTDFTLTISSLEPEDFATYFCQQSWNDPYTFGQGTKLEIK

SEQ ID NO: 139 - protein, 117 aa, synthetic construct
  source 1..117: note = anti-CD30 antibody VH
QIQLQQSGPEVVKPGASVKISCKASGYTFTDYYITWVKQKPGQGLEWIGWIYPGSGNTKYNEKFKGKATLTVDTSSSTAFMQLSSLTSEDTAVYFCANYGNYWFAYWGQGTQVTVSA

SEQ ID NO: 140 - protein, 111 aa, synthetic construct
  source 1..111: note = anti-CD30 antibody VL
DIVLTQSPASLAVSLGQRATISCKASQSVDFDGDSYMNWYQQKPGQPPKVLIYAASNLESGIPARFSGSGSGTDFTLNIHPVEEEDAATYYCQQSNEDPWTFGGGTKLEIK

SEQ ID NO: 141 - protein, 118 aa, synthetic construct
  source 1..118: note = anti-CD40L antibody VH
QVQLVQSGAEVQKPGSSVKVSCKASGGTFSNFAFNWVRQVPGQGLEWMGRILPSLDIASYAQKFQDRVTITADKSTSTAYMELSSLRSEDTAMYYCAREVDGGGFDYWGQGTLVTVSS

SEQ ID NO: 142 - protein, 107 aa, synthetic construct
  source 1..107: note = anti-CD40L antibody VL
DIQMTQSPSSLSASVGDRVTITCRASQGISSWLAWYQQKPEKAPKSLIYAASSLQSGVPSRFSGSGSGTDFTLTISSLQPEDFATYYCQQYNSYPFTFGGGTKVEIK

SEQ ID NO: 143 - protein, 473 aa, Synthetic construct
  source 1..473: note = TRBV50003 VH
QVQLQESGAGLLKPSETLSLTCAVYGGSFSGYYWSWIRQPPGKGLEWIGYIYYSGSTNYNPSLKSRVTISVDTSKNQFSLKLSSVTAADTAVYYCAKAPYMMYFDSWGQGTLVTVSSASTKGPSVFPLAPSSKSTSGGTAALGCLVKDYFPEPVTVSWNSGALTSGVHTFPAVLQSSGLYSLSSVVTVPSSSLGTQTYICNVNHKPSNTKVDKRVEPKSCGGGGSQVQLKESGPGLVAPSQSLSITCTVSGFSLTAYGVNWVRQPPGKGLEWLGMIWGDGNTDYNSALKSRLSISKDNSKSQVFLKMNSLQTDDTARYYCARDRVTATLYAMDYWGQGTSVTVSSGGGGSGGGGSGGGGSDIQMTQTTSSLSASLGDRVTITCSASQGISNYLNWYQQKPDGTVKLLIYYTSSLHSGVPSRFSGSGSGTDYSLTISNLEPEDIATYYCQQYSKLPRTFGGGTKVEIKHHHHHH